European Patent Application EP 4 722 246 A1, published April 8, 2026. Title: 一种靶向TEM8的抗体或其抗原结合片段及其应用. Applicant: 应世生物科技（南京）有限公司. The sequence listing filed with the application follows.

SEQUENCE LISTING (75 sequences)

SEQ ID NO: 1 - protein, 121 aa, artificial sequence
QVQLVQSGPEVKKPGAPVKISCKTSGYIFDDYGITWVRQAPGQGLEWLGWISTYNGKTSFAQKVQGRLTMTTDISTNTASMELRGLRSDDTALYYCARVFSRYIPFYFDSWGQGTLVTVSS

SEQ ID NO: 2 - protein, 113 aa, artificial sequence
DVVMTQSPDSLAVSLGERATINCKSSQSVLYSYNNKNYLAWYQQKPGQPPKLLIYWASTRESGVPDRFSGSGSGTDFTLTISSLQAEDVAVYYCQQYYSTPLTFGGGTKLEIK

SEQ ID NO: 3 - protein, 8 aa, artificial sequence
GYIFDDYG

SEQ ID NO: 4 - protein, 8 aa, artificial sequence
ISTYNGKT

SEQ ID NO: 5 - protein, 14 aa, artificial sequence
ARVFSRYIPFYFDS

SEQ ID NO: 6 - protein, 12 aa, artificial sequence
QSVLYSYNNKNY

SEQ ID NO: 7 - skipped

SEQ ID NO: 8 - protein, 9 aa, artificial sequence
QQYYSTPLT

SEQ ID NO: 9 - protein, 5 aa, artificial sequence
DYGIT

SEQ ID NO: 10 - protein, 17 aa, artificial sequence
WISTYNGKTSFAQKVQG

SEQ ID NO: 11 - protein, 12 aa, artificial sequence
VFSRYIPFYFDS

SEQ ID NO: 12 - protein, 17 aa, artificial sequence
KSSQSVLYSYNNKNYLA

SEQ ID NO: 13 - protein, 7 aa, artificial sequence
WASTRES

SEQ ID NO: 14 - protein, 118 aa, artificial sequence
EVQLVQSGGGLVKPGGSLRLSCAASGFTFSSYSMNWVRQAPGKGLEWVSSISSSSSYIYYADSVKGRFTISRDNAKNSLYLQMNSLRAEDTAVYYCARVRPPYGMDVWGQGTLVTVSS

SEQ ID NO: 15 - protein, 107 aa, artificial sequence
NIQMTQSPSSVSASVGDTVTISCRASQGISNWLGWYQQRPGEAPKLLIYAASHLQSGVPSRFSGSGSGTDFVLTITSLQPEDFATYYCQQSNSFPLAFGGGTKLEIK

SEQ ID NO: 16 - protein, 8 aa, artificial sequence
GFTFSSYS

SEQ ID NO: 17 - protein, 8 aa, artificial sequence
ISSSSSYI

SEQ ID NO: 18 - protein, 11 aa, artificial sequence
ARVRPPYGMDV

SEQ ID NO: 19 - protein, 6 aa, artificial sequence
QGISNW

SEQ ID NO: 20 - skipped

SEQ ID NO: 21 - protein, 9 aa, artificial sequence
QQSNSFPLA

SEQ ID NO: 22 - protein, 5 aa, artificial sequence
SYSMN

SEQ ID NO: 23 - protein, 17 aa, artificial sequence
SISSSSSYIYYADSVKG

SEQ ID NO: 24 - protein, 9 aa, artificial sequence
VRPPYGMDV

SEQ ID NO: 25 - protein, 11 aa, artificial sequence
RASQGISNWLG

SEQ ID NO: 26 - protein, 7 aa, artificial sequence
AASHLQS

SEQ ID NO: 27 - protein, 123 aa, artificial sequence
EVQLVESGGGVVQPGGSLRLSCAASGFTFDDYAMHWVRQAPGKGLEWVSLISGDGGSTYYADSVKGRFTISRDNSKNSLYLQMNSLKASDTAMYYCARPRWGRYSSSWPFDYWGQGTLVTVSS

SEQ ID NO: 28 - protein, 110 aa, artificial sequence
QSALTQPASVSGSPGQSITISCTGTSSDVGTYNYVSWYQQHPGKAPKLMIYDVTDRPSGISNRFSGSKSGNTASLTISGLQAEDEGNYYCSSYTSNRSWVFGGGTKLTVL

SEQ ID NO: 29 - protein, 8 aa, artificial sequence
GFTFDDYA

SEQ ID NO: 30 - protein, 8 aa, artificial sequence
ISGDGGST

SEQ ID NO: 31 - protein, 16 aa, artificial sequence
ARPRWGRYSSSWPFDY

SEQ ID NO: 32 - protein, 9 aa, artificial sequence
SSDVGTYNY

SEQ ID NO: 33 - skipped

SEQ ID NO: 34 - protein, 10 aa, artificial sequence
SSYTSNRSWV

SEQ ID NO: 35 - protein, 5 aa, artificial sequence
DYAMH

SEQ ID NO: 36 - protein, 17 aa, artificial sequence
LISGDGGSTYYADSVKG

SEQ ID NO: 37 - protein, 14 aa, artificial sequence
PRWGRYSSSWPFDY

SEQ ID NO: 38 - protein, 14 aa, artificial sequence
TGTSSDVGTYNYVS

SEQ ID NO: 39 - protein, 7 aa, artificial sequence
DVTDRPS

SEQ ID NO: 40 - protein, 110 aa, artificial sequence
QSALTQPASVSGSPGQSITISCTGTSSDVGTYNYVSWYQQHPGKAPKLMIYDVTDRPSGISNRFSGSKSGNTASLTISGLQAEDEGNYYCSSYTSQRSWVFGGGTKLTVL

SEQ ID NO: 41 - protein, 10 aa, artificial sequence
SSYTSQRSWV

SEQ ID NO: 42 - protein, 122 aa, artificial sequence
QVQLVESGGGLVNPGGSLRLSCAVSGFTSSGFSINWVRQAPGKGLEWVSSISGIGDSIFYADSVKGRFTISRDNAKNLVFLQMNSVKAEDTAVYYCVRDKWGWGTYSLFDYWGQGTLVTVSS

SEQ ID NO: 43 - protein, 110 aa, artificial sequence
QAVLTQPPSASGTPGQRVTISCSGSSSNIASNVVSWYQQLPGTAPKVLIYSNNRRPSGVPDRFSGSKSGASASLAISGLQSDDETHYYCAAWDDSLKGPVFGGGTQLTVL

SEQ ID NO: 44 - protein, 8 aa, artificial sequence
GFTSSGFS

SEQ ID NO: 45 - protein, 8 aa, artificial sequence
ISGIGDSI

SEQ ID NO: 46 - protein, 15 aa, artificial sequence
VRDKWGWGTYSLFDY

SEQ ID NO: 47 - protein, 8 aa, artificial sequence
SSNIASNV

SEQ ID NO: 48 - skipped

SEQ ID NO: 49 - protein, 11 aa, artificial sequence
AAWDDSLKGPV

SEQ ID NO: 50 - protein, 5 aa, artificial sequence
GFSIN

SEQ ID NO: 51 - protein, 17 aa, artificial sequence
SISGIGDSIFYADSVKG

SEQ ID NO: 52 - protein, 13 aa, artificial sequence
DKWGWGTYSLFDY

SEQ ID NO: 53 - protein, 13 aa, artificial sequence
SGSSSNIASNVVS

SEQ ID NO: 54 - protein, 7 aa, artificial sequence
SNNRRPS

SEQ ID NO: 55 - protein, 126 aa, artificial sequence
QVQLVQSGGGVVQPGRPLRLSCAASGFNLGSYAMSWVRQAPGKGLEWVSAISGSGGSTYYADSVKGRFTISRDNSKNTLYLQMNSLRAEDTAVYYCAKILGPGNLNYYYYYGMDVWGQGTTVTVSS

SEQ ID NO: 56 - protein, 108 aa, artificial sequence
SSELTQDPAVSVALGQTVRITCQGDSLRNSYASWYQQKPGQAPVLVIYGNNNRPSGIPDRVSGSRSGNTASLTITGAQAEDEADYYCNSRDSSGNHVVFGGGTELTVL

SEQ ID NO: 57 - protein, 8 aa, artificial sequence
GFNLGSYA

SEQ ID NO: 58 - protein, 8 aa, artificial sequence
ISGSGGST

SEQ ID NO: 59 - protein, 19 aa, artificial sequence
AKILGPGNLNYYYYYGMDV

SEQ ID NO: 60 - protein, 6 aa, artificial sequence
SLRNSY

SEQ ID NO: 61 - skipped

SEQ ID NO: 62 - protein, 11 aa, artificial sequence
NSRDSSGNHVV

SEQ ID NO: 63 - protein, 5 aa, artificial sequence
SYAMS

SEQ ID NO: 64 - protein, 17 aa, artificial sequence
AISGSGGSTYYADSVKG

SEQ ID NO: 65 - protein, 17 aa, artificial sequence
ILGPGNLNYYYYYGMDV

SEQ ID NO: 66 - protein, 11 aa, artificial sequence
QGDSLRNSYAS

SEQ ID NO: 67 - protein, 7 aa, artificial sequence
GNNNRPS

SEQ ID NO: 68 - protein, 532 aa, artificial sequence
EDGGPACYGGFDLYFILDKSGSVLHHWNEIYYFVEQLAHKFISPQLRMSFIVFSTRGTTLMKLTEDREQIRQGLEELQKVLPGGDTYMHEGFERASEQIYYENRQGYRTASVIIALTDGELHEDLFFYSEREANRSRDLGAIVYCVGVKDFNETQLARIADSKDHVFPVNDGFQALQGIIHSILKKSCIEILAAEPSTICAGESFQVVVRGNGFRHARNVDRVLCSFKINDSVTLNEKPFSVEDTYLLCPAPILKEVGMKAALQVSMNDGLSFISSSVIITTTHCSDGSILAIALLILFLLLALALLWWFWPLCCTVIIKEVPPPPAEESEEEDDDGLPKKKWPTVDASYYGGRGVGGIKRMEVRWGEKGSTEEGAKLEKAKNARVKMPEQEYEFPEPRNLNNNMRRPSSPRKWYSPIKGKLDALWVLLRKGYDRVSVMRPQPGDTGRCINFTRVKNNQPAKYPLNNAYHTSSPPPAPIYTPPPPAPHCPPPPPSAPTPPIPSPPSTLPPPPQAPPPNRAPPPSRPPPRPSV

SEQ ID NO: 69 - protein, 532 aa, artificial sequence
EDGGPACYGGFDLYFILDKSGSVLHHWNEIYYFVEQLAHRFISPQLRMSFIVFSTRGTTLMKLTEDREQIRQGLEELQKVLPGGDTYMHEGFERASEQIYYENSQGYRTASVIIALTDGELHEDLFFYSEREANRSRDLGAIVYCVGVKDFNETQLARIADSKDHVFPVNDGFQALQGIIHSILKKSCIEILAAEPSTICAGESFQVVVRGNGFRHARNVDRVLCSFKINDSVTLNEKPFAVEDTYLLCPAPILKEVGMKAALQVSMNDGLSFISSSVIITTTHCSDGSILAIALLVLFLLLALALLWWFWPLCCTVIIKEVPPPPVEESEEEDDDGLPKKKWPTVDASYYGGRGVGGIKRMEVRWGEKGSTEEGAKLEKAKNARVKMPEQEYEFPEPRNLNNNMRRPSSPRKWYSPIKGKLDALWVLLRKGYDRVSVMRPQPGDTGRCINFTRVKNSQPAKYPLNNTYHPSSPPPAPIYTPPPPAPHCPPPAPSAPTPPIPSPPSTLPPPPQAPPPNRAPPPSRPPPRPSV

SEQ ID NO: 70 - protein, 532 aa, artificial sequence
EDAGAACYGGFDLYFILDKSGSVLHHWNEIYYFVEQLAHKFISPQLRMSFIVFSTRGTTLMKLTEDREQIRQGLEELQKVLPGGDTYMHEGFERASEQIYYENSQGYRTASVIIALTDGELHEDLFFYSEREANRSRDLGAIVYCVGVKDFNETQLARIADSKDHVFPVNDGFQALQGIIHSILKKSCIEILAAEPSTICAGESFQVVVRGNGFRHARNVDRVLCSFKINESVTLNEKPFTVEDTYLLCPAPILKEVGMKAALQVSMNDGLSFISSSVIITTTRCSDGSILAIALLILFLLLALALLWWFWPLCCTVIIKEVPPPPAEESEEEDDDGLPKKKWPTVDASYYGGRGVGGIKRMEVRWGEKGSTEEGAKLEKAKNARVKMPEQEYEFPEPRNLNNNLRRPSSPRKWYSPIKGKLDALWVLLRKGYDRVSVMRPQPGDTGRCINFTRVKNNQPAKYPLNNAYHTSSPPPAPIYTPPPPAPHCPPPPPSAPTPPIPSPPSTLPPPPHAPPPSRAPPPSRPPPRPSV

SEQ ID NO: 71 - protein, 330 aa, artificial sequence
ASTKGPSVFPLAPSSKSTSGGTAALGCLVKDYFPEPVTVSWNSGALTSGVHTFPAVLQSSGLYSLSSVVTVPSSSLGTQTYICNVNHKPSNTKVDKKVEPKSCDKTHTCPPCPAPEAAGGPSVFLFPPKPKDTLMISRTPEVTCVVVDVSHEDPEVKFNWYVDGVEVHNAKTKPREEQYNSTYRVVSVLTVLHQDWLNGKEYKCKVSNKALGAPIEKTISKAKGQPREPQVYTLPPSRDELTKNQVSLTCLVKGFYPSDIAVEWESNGQPENNYKTTPPVLDSDGSFFLYSKLTVDKSRWQQGNVFSCSVMHEALHNHYTQKSLSLSPGK

SEQ ID NO: 72 - protein, 107 aa, artificial sequence [sequence omitted]

SEQ ID NO: 73 - protein, 106 aa, artificial sequence
GQPKAAPSVTLFPPSSEELQANKATLVCLISDFYPGAVTVAWKADSSPVKAGVETTTPSKQSNNKYAASSYLSLTPEQWKSHRSYSCQVTHEGSTVEKTVAPTECS

SEQ ID NO: 74 - protein, 447 aa, artificial sequence
QVQLKESGPALVKPTQTLTLTCTFSGFSLSTSGGGVSWIRQPPGKALEWLAHIYSNDDKSYSTSLKTRLTISKDTSKNQVVLTMTNMDPVDTATYYCARGGYFLDYWGQGTLVTVSSASTKGPSVFPLAPSSKSTSGGTAALGCLVKDYFPEPVTVSWNSGALTSGVHTFPAVLQSSGLYSLSSVVTVPSSSLGTQTYICNVNHKPSNTKVDKKVEPKSCDKTHTCPPCPAPELLGGPSVFLFPPKPKDTLMISRTPEVTCVVVDVSHEDPEVKFNWYVDGVEVHNAKTKPREEQYNSTYRVVSVLTVLHQDWLNGKEYKCKVSNKALPAPIEKTISKAKGQPREPQVYTLPPSRDELTKNQVSLTCLVKGFYPSDIAVEWESNGQPENNYKTTPPVLDSDGSFFLYSKLTVDKSRWQQGNVFSCSVMHEALHNHYTQKSLSLSPGK

SEQ ID NO: 75 - protein, 212 aa, artificial sequence
DIELTQPPSVSVAPGQTARISCSGDNIGGIYVHWYQQKPGQAPVLVIYADSKRPSGIPERFSGSNSGNTATLTISGTQAEDEADYYCQSYDITSLVFGGGTKLTVLGQPKAAPSVTLFPPSSEELQANKATLVCLISDFYPGAVTVAWKADSSPVKAGVETTTPSKQSNNKYAASSYLSLTPEQWKSHRSYSCQVTHEGSTVEKTVAPTECS